European Patent Specification EP 3 704 136 B1, published December 4, 2024. Title: Adapter-based retroviral vector system for the selective transduction of target cells. Applicant: Miltenyi Biotec GmbH. The sequence listing filed with the application follows.

SEQUENCE LISTING (15 sequences)

SEQ ID NO: 1 - protein, 122 aa, Artificial sequence
  Biotin AB heavy chain
EVQLVESGGGLVKPGGSLKLSCAVSGFTFSNYAMSWVRQTPETRLNWVATITGGGSYTYYPDSVKGRFTISRDNAKDTLYLQMSSLRSEDTAMYYCVRQRVGDYVSSLLGYWGQGTLVTVSA

SEQ ID NO: 2 - protein, 112 aa, Artificial sequence
  Biotin AB light chain
DVVMTQTPLSLPVSLGDQASISCRSSQSLVHSNGNTYLHWFLQKPGQSPNLLIYKVSNRFSGVPDRFSGSGSGTDFTLKISRVEAEDLGVYFCSQSTHVPYTFGGGTKLEIK

SEQ ID NO: 3 - protein, 5 aa, Artificial sequence
  measles virus (Edmonston strain); transmembrane domain of F protein
LICCC

SEQ ID NO: 4 - protein, 4 aa, Artificial sequence
  measles virus (Edmonston strain); transmembrane domain of H protein
PYVL

SEQ ID NO: 5 - protein, 33 aa, Artificial sequence
  measles virus (Edmonston strain); cytoplasmic domain of F protein
RGRCNKKGEQVGMSRPGLKPDLTGTSKSYVRSL

SEQ ID NO: 6 - protein, 34 aa, Artificial sequence
  measles virus (Edmonston strain); cytoplasmic domain of H protein
MSPQRDRINAFYKDNPHPKGSRIVINREHLMIDR

SEQ ID NO: 7 - protein, 21 aa, Artificial sequence
  Nipah Virus; transmembrane domain of G protein
FNTYIALLGSIVIIVMNIMII

SEQ ID NO: 8 - protein, 45 aa, Artificial sequence
  Nipah Virus; cytoplasmic domain of G protein
MPAENKKVRFENTTSDKGKIPSKVIKSYYGTMDIKKINEGLLDSK

SEQ ID NO: 9 - protein, 21 aa, Artificial sequence
  Nipah Virus; transmembrane domain of F protein
YVLSIASLCIGLITFISFIIV

SEQ ID NO: 10 - protein, 28 aa, Artificial sequence
  Nipah Virus; cytoplasmic domain of F protein
EKKRNTYSRLEDRRVRPTSSGDLYYIGT

SEQ ID NO: 11 - protein, 15 aa, Artificial sequence
  scFV linker sequence
GGGGSGGGGSGGGGS

SEQ ID NO: 12 - protein, 6 aa, Artificial sequence
  HIS tag sequence
HHHHHH

SEQ ID NO: 13 - protein, 117 aa, Artificial sequence
  Dextran AB heavy chain
EVQLQQSGPELVKPGASVKISCKASGYTFTDYYMNWVKQSHGKSLEWIGDINPNNGGTSYNQKFKGKATLTVDKSSSTAYMELRSLTSEDSAVYYCAPYYYTSSLVWGTGTTVTVSA

SEQ ID NO: 14 - protein, 106 aa, Artificial sequence
  Dextran AB light chain
QIVLTQSPAIMSASPGEKVTMTCSASSSVSYMHWYQQKSGTSPKRWIYDTSKLASGVPARFSGSGSGTSYSLTISSMEAEDAATYYCQQWSSNPLTFGAGTKLELK

SEQ ID NO: 15 - protein, 26 aa, Artificial sequence
  Vectofusin
KKALLALALHHLAHLALHLALALKKA